European Patent Specification EP 3 621 693 B1, published June 24, 2026. Title: Anti-IL-1R3 antibodies for use in inflammatory conditions. Applicant: MAB Discovery GmbH. Application EP 17169953. The sequence listing filed with the application follows.

SEQUENCE LISTING (183 sequences)

SEQ ID NO: 1 - protein, 118 aa, Artificial Sequence
  humanized antibody
EVQLEESGGGLVQPGGSLRLSCAASGFSFSSSYWICWVRQAPGKGLEWVSCIYTGSGGTYYASWEKGRFTISRDNSKNTLYLQMNSLRAEDTAVYFCARDPGYSSWLWGQGTLVTVSS

SEQ ID NO: 2 - protein, 122 aa, Artificial Sequence
  humanized antibody
EVQLEESGGDLVQPGGSLRLSCAASGFSFSSSHYMCWVRQAPGKGLEWVSCIYAGSSGNTYYANWAKGRFTISRDNSKNTLYLQMNSLRAEDTAVYFCARVDASSSGSWDLWGQGTLVTVSS

SEQ ID NO: 3 - protein, 123 aa, Artificial Sequence
  humanized antibody
EVQLEESGGRLVQPGGSLRLSCAVSGIDLSSYAMGWVRQAPGKGLEYVSVITSSATTYYASWAKGRFTISRDNSKNTLYLQMNSLRAEDTAVYFCARGGPGYSTNTHYAFDPWGQGTLVTVSS

SEQ ID NO: 4 - protein, 119 aa, Artificial Sequence
  humanized antibody
EVQLEESGGRVVQPGRSLRLSCAVSGIDLDNYAMGWVRQAPGKGLEYVAVISSDGFFYDASWAKGRFTISRDNSKNTLYLQMNSLRAEDTAVYFCARDRGTSTGSLDLWGQGTLVTVSS

SEQ ID NO: 5 - protein, 125 aa, Artificial Sequence
  humanized antibody
EVQLEESGGRLVQPGGSLRLSCAASGFSLSSYYMSWVRQAPGKGLEWVSIISGSASTYYATWAKGRFTISRDNSKNTLYLQMNSLRAEDTAVYFCARTHYAAVAGYGYASRLDLWGQGTLVTVSS

SEQ ID NO: 6 - protein, 120 aa, Artificial Sequence
  humanized antibody
EVQLEESGGDLVQPGGSLRLSCAASGFSFSSNYWICWVRQAPGKGLELVSCIYTSTGNTWYASWAKGRFTISRDNSKNTLYLQMNSLRAEDTAVYFCARDLLVVTSFNLWGQGTLVTVSS

SEQ ID NO: 7 - protein, 120 aa, Artificial Sequence
  humanized antibody
EVQLEESGGDLVQPGGSLRLSCAASGFSFSSSYYMCWVRQAPGKGLEWVSCIYAGSSGVTYYASWAKGRFTISRDNSKNTLYLQMNSLRAEDTAVYFCASETDGNYFNLWGQGTLVTVSS

SEQ ID NO: 8 - protein, 120 aa, Artificial Sequence
  humanized antibody
EVQLEQSGGGLVQPGGSLRLSCAASGFSLSTSYWRCWVRQAPGKGLEWVSCIYAGSGDVTYYANWVNGRFTISRDNSKNTLYLQMNSLRAEDTAVYYCASGVGFGYFNLWGQGTLVTVSS

SEQ ID NO: 9 - protein, 122 aa, Artificial Sequence
  humanized antibody
EVQLEESGGGLVQPGGSLRLSCAASGIDFSSYYYMCWVRQAPGKGLEWVSCIFIGYGDVTWYASWAKGRFTISRDNSKNTLYLQMNSLRAEDTAVYFCARALGSSGYRVNLWGQGTLVTVSS

SEQ ID NO: 10 - protein, 115 aa, Artificial Sequence
  humanized antibody
EVQLEESGGRLVQPGGSLRLSCAASGFSLSSYWMSWVRQAPGKGLEWVSMIYGSGYTYYASWAKGRFTISRDNSKNTLYLQMNSLRAEDTAVYFCARDPQYFILWGQGTLVTVSS

SEQ ID NO: 11 - protein, 120 aa, Artificial Sequence
  humanized antibody
EVQLEESGGRLVQPGGSLRLSCAVSGFSLSSYDMSWVRQAPGKGLEWVSTIYIGGTTAYASWPKGRFTISRDNSKNTLYLQMNSLRAEDTAVYFCARLQGANYYNSLALWGQGTLVTVSS

SEQ ID NO: 12 - protein, 120 aa, Artificial Sequence
  humanized antibody
EVQLVESGGGLVQPGGSLRLSCAASGFDFSSNYYMCWVRQAPGKGLELVSCIYTNSGNTWSASWAKGRFTISRDNSKNTLYLQMNSLRAEDTAVYFCARDLNYPDTSNLWGQGTLVTVSS

SEQ ID NO: 13 - protein, 119 aa, Artificial Sequence
  humanized antibody
EVQLEESGGDLVQPGGSLRLSCAASGFSFSFGYYMCWVRQAPGKGLEWVSCIYGDSSDTLYANWAKGRFTISRDNSKNTLYLQMNSLRAEDTAVYFCARYPGGSYYNLWGQGTLVTVSS

SEQ ID NO: 14 - protein, 122 aa, Artificial Sequence
  humanized antibody
EVQLEESGGDLVQPGGSLRLSCAASGFSFSSTYYMCWVRQAPGKGLEWVSCIYAGSSGSTYYASWAKGRFTISRDNSKNTLYLQMNSLRAEDTAVYFCARVDGSSSGSWDLWGQGTLVTVSS

SEQ ID NO: 15 - protein, 122 aa, Artificial Sequence
  humanized antibody
EVQLEESGGDLVQPGGSLRLSCAASGISFSSSDFMCWVRQAPGKGLEWVSCIYAGSSVSIYYATWAKGRFTISRDNSKNTLYLQMNSLRAEDTAVYFCARSTGSVGRGFNLWGQGTLVTVSS

SEQ ID NO: 16 - protein, 121 aa, Artificial Sequence
  humanized antibody
EVQLVESGGGLVQPGGSLRLSCAASGFSFSSIYYMCWVRQAPGKGLEWVSCIYTGNSDFTYYANWAKGRFTISRDNSKNTLYLQMNSLRAEDTAVYFCARFRDDYASLKLWGQGTLVTVSS

SEQ ID NO: 17 - protein, 120 aa, Artificial Sequence
  humanized antibody
EVQLEESGGGLVQPGGSLRLSCAASGFSFSSGYDMCWVRQAPGKGLEWVSCIYTGSGSTYYANWAKGRFTISRDNSKNTLYLQMNSLRAEDTAVYFCARNSNDWMYFNLWGQGTLVTVSS

SEQ ID NO: 18 - protein, 117 aa, Artificial Sequence
  humanized antibody
EVQLEQSGGGLVQPGGSLRLSCAASGFSFSSSYWICWVRQAPGKGLEWVACIYTGSGGTYYASWEKGRFTISKTSSTTLYLQMNSLRAEDTAVYFCARDPGYSSWLWGQGTLVTVSS

SEQ ID NO: 19 - protein, 122 aa, Artificial Sequence
  humanized antibody
EVQLEESGGDLVQPGASLRLSCAASGFSFSSSHYMCWVRQAPGKGLEWVACIYAGSSGNTYYANWAKGRFTISKTNSKNTLYLQMNSLRAEDTAVYFCARVDASSSGSWDLWGQGTLVTVSS

SEQ ID NO: 20 - protein, 122 aa, Artificial Sequence
  humanized antibody
EVQLLESGGRLVQPGTSLRLSCAVSGIDLSSYAMGWVRQAPGKGLEYVGVITSSATTYYASWAKGRFTISKTSSTTLYLQMNSLRAEDTAVYFCARGGPGYSTNTHYAFDPWGQGTLVTVSS

SEQ ID NO: 21 - protein, 119 aa, Artificial Sequence
  humanized antibody
EVQLEESGGRVVQPGTSLRLSCAVSGIDLDNYAMGWVRQAPGKGLEYVAVISSDGFFYDASWAKGRFTISKANSKNTLYLQMNSLRAEDTAVYFCARDRGTSTGSLDLWGQGTLVTVSS

SEQ ID NO: 22 - protein, 123 aa, Artificial Sequence
  humanized antibody
QVQLEESGGRLVQPGTSLRLSCAASGFSLSSYYMSWVRQAPGKGLEWVAIISGSASTYYATWAKGRFTISKTSTTLYLQMNSLRAEDTAVYFCARTHYAAVAGYGYASRLDLWGQGTLVTVSS

SEQ ID NO: 23 - protein, 120 aa, Artificial Sequence
  humanized antibody
QVQLQESGGDLVQPGGSLRLSCAASGFSFSSNYWICWVRQAPGKGLELVACIYTSTGNTWYASWAKGRFTISRDNSKNTLYLQMNSLRAEDTAVYFCARDLLVVTSFNLWGQGTLVTVSS

SEQ ID NO: 24 - protein, 119 aa, Artificial Sequence
  humanized antibody
EVQLVESGGDLVQPGASLRLSCAASGFSFSSSYYMCWVRQAPGKGLEWVACIYAGSSGVTYYASWAKGRFTISDTSSTTLYLQMNSLRAEDTAVYFCASETDGNYFNLWGQGTLVTVSS

SEQ ID NO: 25 - protein, 120 aa, Artificial Sequence
  humanized antibody
EVQLEQSGGGLVQPGGSLRLSCAASGFSLSTSYWRCWVRQAPGKGLEWVACIYAGSGDVTYYANWVNGRFTISRDNSKSTLYLQMNSLRAEDTAVYYCASGVGFGYFNLWGQGTLVTVSS

SEQ ID NO: 26 - protein, 122 aa, Artificial Sequence
  humanized antibody
EVQLEESGGGLVQPGGSLRLSCAASGIDFSSYYYMCWVRQAPGKGLEWVACIFIGYGDVTWYASWAKGRFTISKANSKNTLYLQMNSLRAEDTAVYFCARALGSSGYRVNLWGQGTLVTVSS

SEQ ID NO: 27 - protein, 113 aa, Artificial Sequence
  humanized antibody
QVQLEESGGRLVQPGASLRLSCAASGFSLSSYWMSWVRQAPGKGLEWVAMIYGSGYTYYASWAKGRFTISTTSTTLYLQMNSLRAEDTAVYFCARDPQYFILWGQGTLVTVSS

SEQ ID NO: 28 - protein, 120 aa, Artificial Sequence
  humanized antibody
EVQLEESGGRLVQPGTSLRLSCAVSGFSLSSYDMSWVRQAPGKGLEWVSTIYIGGTTAYASWPKGRFTISKTNSKNTLYLQMNSLRAEDTAVYFCARLQGANYYNSLALWGQGTLVTVSS

SEQ ID NO: 29 - protein, 119 aa, Artificial Sequence
  humanized antibody
QVQLVESGGGLVQPGGSLRLSCAASGFDFSSNYYMCWVRQAPGKGLELVACIYTNSGNTWSASWAKGRFTISKTNSTTLYLQMNSLRAEDTAVYFCARDLNYPDTSNLWGQGTLVTVSS

SEQ ID NO: 30 - protein, 119 aa, Artificial Sequence
  humanized antibody
EVQLEESGGDLVQPGGSLRLSCAASGFSFSFGYYMCWVRQAPGKGLEWVACIYGDSSDTLYANWAKGRFTISKTNSKNTLYLQMNSLRAEDTAVYFCARYPGGSYYNLWGQGTLVTVSS

SEQ ID NO: 31 - protein, 120 aa, Artificial Sequence
  humanized antibody
QVQLQESGGDLVQPGASLRLSCAASGFSFSSTYYMCWVRQAPGKGLEWVACIYAGSSGSTYYASWAKGRFTISKNSSTLYLQMNSLRAEDTAVYFCARVDGSSSGSWDLWGQGTLVTVSS

SEQ ID NO: 32 - protein, 121 aa, Artificial Sequence
  humanized antibody
EVQLEESGGDLVQPGASLRLSCAASGISFSSSDFMCWVRQAPGKGLEWVACIYAGSSVSIYYATWAKGRFTISKASSTTLYLQMNSLRAEDTAVYFCARSTGSVGRGFNLWGQGTLVTVSS

SEQ ID NO: 33 - protein, 121 aa, Artificial Sequence
  humanized antibody
EVQLVESGGGLVQPGGSLRLSCAASGFSFSSIYYMCWVRQAPGKGLEWVGCIYTGNSDFTYYANWAKGRFTISRDNSKSTLYLQMNSLRAEDTAVYFCARFRDDYASLKLWGQGTLVTVSS

SEQ ID NO: 34 - protein, 120 aa, Artificial Sequence
  humanized antibody
QVQLQESGGGLVQPGGSLRLSCTASGFSFSSGYDMCWVRQAPGKGLEWVGCIYTGSGSTYYANWAKGRFTISKDNSKTTLYLQMNSLRAEDTAVYFCARNSNDWMYFNLWGQGTLVTVSS

SEQ ID NO: 35 - protein, 110 aa, Artificial Sequence
  humanized antibody
DIVMTQSPSSLSASVGDRVTITCQASESISNYLSWYQQKPGQAPKLLIYLASTLASGVPSRFSGSGSGTDFTLTISSLQPEDFATYYCQNWWVIEHNGAAFGGGTKVVIK

SEQ ID NO: 36 - protein, 110 aa, Artificial Sequence
  humanized antibody
DIQMTQSPSSLSASVGDRVTITCQASESIYSNLAWYQQKPGQAPKLLIYAASLLASGVPSRFSGSGSGTDFTLTISSLQPEDFATYYCQSASYSTGPDWTFGQGTKVVIK

SEQ ID NO: 37 - protein, 110 aa, Artificial Sequence
  humanized antibody
DIQMTQSPSSLSASVGDRVTITCQASQSIYIYLSWYQQKPGQAPKLLIYDASKLASGVPSRFSGSGSGTDFTLTISSLQPEDFATYYCQQGATTYNVDNVFGQGTKVVIK

SEQ ID NO: 38 - protein, 111 aa, Artificial Sequence
  humanized antibody
DIVMTQSPSSLSASVGDRVTITCQASENIGNGLAWYQQKPGQAPKLLIYGASTLASGVPSRFSGSGSGTDFTLTISSLQPEDFATYYCQCTYWNPDYIGGAFGGGTKVVIK

SEQ ID NO: 39 - protein, 110 aa, Artificial Sequence
  humanized antibody
DIQMTQSPSSLSASVGDRVTITCLASEDIYSGISWYQQKPGKAPKLLIYAASNLESGVPSRFSGSGSGTDFTLTISSLQPEDFATYYCLGGYSYSNTGPTFGQGTKVEIK

SEQ ID NO: 40 - protein, 113 aa, Artificial Sequence
  humanized antibody
DIVMTQSPSSLSASVGDRVTITCQASEDIYSNLAWFQQKPGQAPKLLIYGASTLASGVPSRFSGSGSGTEFTLTISSLQPEDFATYYCLGVCTDISTDDLYNAFGQGTKVVIK

SEQ ID NO: 41 - protein, 110 aa, Artificial Sequence
  humanized antibody
DIVMTQSPSSLSASVGDRVTITCQASEDIYSNLAWFQQKPGQAPKLLIYRASTLASGVPSRFSGSGSGTEFTLTISSLQPEDFATYYCLGVYTYSTDIHAFGGGTKVVIK

SEQ ID NO: 42 - protein, 110 aa, Artificial Sequence
  humanized antibody
DIVMTQSPSSLSASVGDRVTITCQASEDIYSNLAWFQQKPGQAPKLLIYDASTLASGVPSRFSGSGSGTEFTLTISSLQPEDFATYYCLGVYTHISADNAFGGGTKVVIK

SEQ ID NO: 43 - protein, 111 aa, Artificial Sequence
  humanized antibody
DIQMTQSPSSLSASVGDRVTITCQASENIYSSLAWYQQKPGQAPKLLIYDASDLASGVPSRFSGSGSGTDFTLTISSLQPEDFATYYCQQGYYSGGTDNDVFGGGTKVVIK

SEQ ID NO: 44 - protein, 112 aa, Artificial Sequence
  humanized antibody
DIVMTQSPSSLSASVGDRVTITCQSSQSVDGNNLLSWYQQKPGQAPKLLIYDASNLASGVPSRFSGSGSGTDFTLTISSLQPEDFATYYCQGSYYSSSWYNVFGQGTKVVIK

SEQ ID NO: 45 - protein, 108 aa, Artificial Sequence
  humanized antibody
DIQMTQSPSSLSASVGDRVTITCQASQSIYSFLSWYQQKPGQAPKLLIYAASDLESGVPSRFSGSGSGTDFTLTISSLQPEDFATYYCQCNYIIDYGAFGQGTKVVIK

SEQ ID NO: 46 - protein, 108 aa, Artificial Sequence
  humanized antibody
DIQMTQSPSSLSASVGDRVTITCQASQSIGYYLAWYQQKPGQAPKLLIYRASTLASGVPSRFSGSGSGTDFTLTISSLQPEDFATYYCQSYYNSDSDAFGQGTKVVIK

SEQ ID NO: 47 - protein, 110 aa, Artificial Sequence
  humanized antibody
DIVMTQSPSSLSASVGDRVTITCQASQTISINLAWYQQKPGQAPKLLIYYASTLASGVPSRFSGSGSGTDFTLTISSLQPEDFATYYCQQGYTEDNIDNTFGQGTKVVIK

SEQ ID NO: 48 - protein, 110 aa, Artificial Sequence
  humanized antibody
DIQMTQSPSSLSASVGDRVTITCQASQNIYSNLAWYQQKPGQAPKLLIYAASLLASGVPSRFSGSGSGTDFTLTISSLQPEDFATYYCQGAVYSGNTEWAFGQGTKVVIK

SEQ ID NO: 49 - protein, 113 aa, Artificial Sequence
  humanized antibody
DIVMTQSPSSLSASVGDRVTITCQASQSVYNSNHLSWYQQKPGQAPKLLIYSASTLASGVPSRFSGSGSGTDFTLTISSLQPEDFATYYCQGEFSCVSADCIAFGGGTKVVIK

SEQ ID NO: 50 - protein, 110 aa, Artificial Sequence
  humanized antibody
DIQMTQSPSSLSASVGDRVTITCQASQSISSYLSWYQQKPGQAPKLLIYGASNLASGVPSRFSGSGSGTDFTLTISSLQPEDFATYYCQCTYYDNNYGGAFGGGTKVVIK

SEQ ID NO: 51 - protein, 114 aa, Artificial Sequence
  humanized antibody
DIVMTQSPSSLSASVGDRVTITCQASESISANYWSWYQQKPGQAPKLLIYGASTLASGVPSRFSGSGSGTDFTLTISSLQPEDFATYFCQSWYYSGSGSYHSWAFGQGTKVVIK

SEQ ID NO: 52 - protein, 110 aa, Artificial Sequence; identical to SEQ ID NO: 35
  humanized antibody

SEQ ID NO: 53 - protein, 110 aa, Artificial Sequence
  humanized antibody
AIQMTQSPSSLSASVGDRVTITCQASESIYSNLAWYQQKPGQAPKLLIYAASLLASGVPSRFSGSGSGTDYTLTISSLQPEDFATYYCQSASYSTGPDWTFGQGTKVVIK

SEQ ID NO: 54 - protein, 110 aa, Artificial Sequence
  humanized antibody
AIRMTQSPSSLSASVGDRVTITCQASQSIYIYLSWYQQKPGQAPKLLIYDASKLASGVPSRFSGSGSGTDFTLTISSLQPEDFATYYCQQGATTYNVDNVFGQGTKVVIK

SEQ ID NO: 55 - protein, 111 aa, Artificial Sequence
  humanized antibody
ELVMTQSPSSLSASVGDRVTITCQASENIGNGLAWYQQKPGQAPKLLIYGASTLASGVPSRFSGSGSGTDFTLTISSLQPEDFATYYCQCTYWNPDYIGGAFGGGTKVVIK

SEQ ID NO: 56 - protein, 110 aa, Artificial Sequence
  humanized antibody
AIQMTQSPSSLSASVGDRVTITCLASEDIYSGISWYQQKPGKAPKLLIYAASNLESGVPSRFSGSGSGTDYTLTISSLQPEDFATYYCLGGYSYSNTGPTFGQGTKVEIK

SEQ ID NO: 57 - protein, 113 aa, Artificial Sequence; identical to SEQ ID NO: 40
  humanized antibody

SEQ ID NO: 58 - protein, 110 aa, Artificial Sequence; identical to SEQ ID NO: 41
  humanized antibody

SEQ ID NO: 59 - protein, 110 aa, Artificial Sequence
  humanized antibody
ELVMTQSPSSLSASVGDRVTITCQASEDIYSNLAWFQQKPGQAPKLLIYDASTLASGVPSRFSGSGSGTEFTLTISSLQPEDFATYYCLGVYTHISADNAFGGGTKVEIK

SEQ ID NO: 60 - protein, 111 aa, Artificial Sequence
  humanized antibody
ALQMTQSPSSLSASVGDRVTITCQASENIYSSLAWYQQKPGQAPKLLIYDASDLASGVPSRFSGSGSGTDFTLTISSLQPEDFATYYCQQGYYSGGTDNDVFGGGTKVVIK

SEQ ID NO: 61 - protein, 112 aa, Artificial Sequence
  humanized antibody
NIVMTQSPSSLSASVGDRVTITCQSSQSVDGNNLLSWYQQKPGQAPKLLIYDASNLASGVPSRFSGSGSGTDFTLTISSLQPEDFATYYCQGSYYSSSWYNVFGQGTKVVIK

SEQ ID NO: 62 - protein, 108 aa, Artificial Sequence
  humanized antibody
DVQMTQSPSSLSASVGDRVTITCQASQSIYSFLSWYQQKPGQAPKLLIYAASDLESGVPSRFSGSGSGTDFTLTISSLQPEDFATYYCQCNYIIDYGAFGQGTKVVIK

SEQ ID NO: 63 - protein, 108 aa, Artificial Sequence; identical to SEQ ID NO: 46
  humanized antibody

SEQ ID NO: 64 - protein, 110 aa, Artificial Sequence
  humanized antibody
AIVMTQSPSSLSASVGDRVTITCQASQTISINLAWYQQKPGQAPKLLIYYASTLASGVPSRFSGSGSGTDFTLTISSLQPEDFATYYCQQGYTEDNIDNTFGQGTKVVIK

SEQ ID NO: 65 - protein, 110 aa, Artificial Sequence
  humanized antibody
AIQMTQSPSSLSASVGDRVTITCQASQNIYSNLAWYQQKPGQAPKLLIYAASLLASGVPSRFSGSGSGTDYTLTISSLQPEDFATYYCQGAVYSGNTEWAFGQGTKVVIK

SEQ ID NO: 66 - protein, 113 aa, Artificial Sequence; identical to SEQ ID NO: 49
  humanized antibody

SEQ ID NO: 67 - protein, 110 aa, Artificial Sequence
  humanized antibody
DVVMTQSPSSLSASVGDRVTITCQASQSISSYLSWYQQKPGQAPKLLIYGASNLASGVPSRFSGSGSGTDFTLTISSLQPEDFATYYCQCTYYDNNYGGAFGGGTKVEIK

SEQ ID NO: 68 - protein, 114 aa, Artificial Sequence; identical to SEQ ID NO: 51
  humanized antibody

SEQ ID NO: 69 - protein, 6 aa, Artificial Sequence
  humanized antibody
SSYWIC

SEQ ID NO: 70 - protein, 6 aa, Artificial Sequence
  humanized antibody
SSHYMC

SEQ ID NO: 71 - protein, 5 aa, Artificial Sequence
  humanized antibody
SYAMG

SEQ ID NO: 72 - protein, 5 aa, Artificial Sequence
  humanized antibody
NYAMG

SEQ ID NO: 73 - protein, 5 aa, Artificial Sequence
  humanized antibody
SYYMS

SEQ ID NO: 74 - protein, 6 aa, Artificial Sequence
  humanized antibody
SNYWIC

SEQ ID NO: 75 - protein, 6 aa, Artificial Sequence
  humanized antibody
SSYYMC

SEQ ID NO: 76 - protein, 6 aa, Artificial Sequence
  humanized antibody
TSYWRC

SEQ ID NO: 77 - protein, 6 aa, Artificial Sequence
  humanized antibody
SYYYMC

SEQ ID NO: 78 - protein, 5 aa, Artificial Sequence
  humanized antibody
SYWMS

SEQ ID NO: 79 - protein, 5 aa, Artificial Sequence
  humanized antibody
SYDMS

SEQ ID NO: 80 - protein, 6 aa, Artificial Sequence
  humanized antibody
SNYYMC

SEQ ID NO: 81 - protein, 6 aa, Artificial Sequence
  humanized antibody
FGYYMC

SEQ ID NO: 82 - protein, 6 aa, Artificial Sequence
  humanized antibody
STYYMC

SEQ ID NO: 83 - protein, 6 aa, Artificial Sequence
  humanized antibody
SSDFMC

SEQ ID NO: 84 - protein, 6 aa, Artificial Sequence
  humanized antibody
SIYYMC

SEQ ID NO: 85 - protein, 6 aa, Artificial Sequence
  humanized antibody
SGYDMC

SEQ ID NO: 86 - protein, 17 aa, Artificial Sequence
  humanized antibody
CIYTGSGGTYYASWEKG

SEQ ID NO: 87 - protein, 18 aa, Artificial Sequence
  humanized antibody
CIYAGSSGNTYYANWAKG

SEQ ID NO: 88 - protein, 16 aa, Artificial Sequence
  humanized antibody
VITSSATTYYASWAKG

SEQ ID NO: 89 - protein, 16 aa, Artificial Sequence
  humanized antibody
VISSDGFFYDASWAKG

SEQ ID NO: 90 - protein, 16 aa, Artificial Sequence
  humanized antibody
IISGSASTYYATWAKG

SEQ ID NO: 91 - protein, 17 aa, Artificial Sequence
  humanized antibody
CIYTSTGNTWYASWAKG

SEQ ID NO: 92 - protein, 18 aa, Artificial Sequence
  humanized antibody
CIYAGSSGVTYYASWAKG

SEQ ID NO: 93 - protein, 18 aa, Artificial Sequence
  humanized antibody
CIYAGSGDVTYYANWVNG

SEQ ID NO: 94 - protein, 18 aa, Artificial Sequence
  humanized antibody
CIFIGYGDVTWYASWAKG

SEQ ID NO: 95 - protein, 16 aa, Artificial Sequence
  humanized antibody
MIYGSGYTYYASWAKG

SEQ ID NO: 96 - protein, 16 aa, Artificial Sequence
  humanized antibody
TIYIGGTTAYASWPKG

SEQ ID NO: 97 - protein, 17 aa, Artificial Sequence
  humanized antibody
CIYTNSGNTWSASWAKG

SEQ ID NO: 98 - protein, 17 aa, Artificial Sequence
  humanized antibody
CIYGDSSDTLYANWAKG

SEQ ID NO: 99 - protein, 18 aa, Artificial Sequence
  humanized antibody
CIYAGSSGSTYYASWAKG

SEQ ID NO: 100 - protein, 18 aa, Artificial Sequence
  humanized antibody
CIYAGSSVSIYYATWAKG

SEQ ID NO: 101 - protein, 18 aa, Artificial Sequence
  humanized antibody
CIYTGNSDFTYYANWAKG

SEQ ID NO: 102 - protein, 17 aa, Artificial Sequence
  humanized antibody
CIYTGSGSTYYANWAKG

SEQ ID NO: 103 - protein, 8 aa, Artificial Sequence
  humanized antibody
DPGYSSWL

SEQ ID NO: 104 - protein, 11 aa, Artificial Sequence
  humanized antibody
VDASSSGSWDL

SEQ ID NO: 105 - protein, 15 aa, Artificial Sequence
  humanized antibody
GGPGYSTNTHYAFDP

SEQ ID NO: 106 - protein, 11 aa, Artificial Sequence
  humanized antibody
DRGTSTGSLDL

SEQ ID NO: 107 - protein, 17 aa, Artificial Sequence
  humanized antibody
THYAAVAGYGYASRLDL

SEQ ID NO: 108 - protein, 10 aa, Artificial Sequence
  humanized antibody
DLLVVTSFNL

SEQ ID NO: 109 - protein, 9 aa, Artificial Sequence
  humanized antibody
ETDGNYFNL

SEQ ID NO: 110 - protein, 9 aa, Artificial Sequence
  humanized antibody
GVGFGYFNL

SEQ ID NO: 111 - protein, 11 aa, Artificial Sequence
  humanized antibody
ALGSSGYRVNL

SEQ ID NO: 112 - protein, 7 aa, Artificial Sequence
  humanized antibody
DPQYFIL

SEQ ID NO: 113 - protein, 12 aa, Artificial Sequence
  humanized antibody
LQGANYYNSLAL

SEQ ID NO: 114 - protein, 10 aa, Artificial Sequence
  humanized antibody
DLNYPDTSNL

SEQ ID NO: 115 - protein, 9 aa, Artificial Sequence
  humanized antibody
YPGGSYYNL

SEQ ID NO: 116 - protein, 11 aa, Artificial Sequence
  humanized antibody
VDGSSSGSWDL

SEQ ID NO: 117 - protein, 11 aa, Artificial Sequence
  humanized antibody
STGSVGRGFNL

SEQ ID NO: 118 - protein, 10 aa, Artificial Sequence
  humanized antibody
FRDDYASLKL

SEQ ID NO: 119 - protein, 10 aa, Artificial Sequence
  humanized antibody
NSNDWMYFNL

SEQ ID NO: 120 - protein, 11 aa, Artificial Sequence
  humanized antibody
QASESISNYLS

SEQ ID NO: 121 - protein, 11 aa, Artificial Sequence
  humanized antibody
QASESIYSNLA

SEQ ID NO: 122 - protein, 11 aa, Artificial Sequence
  humanized antibody
QASQSIYIYLS

SEQ ID NO: 123 - protein, 11 aa, Artificial Sequence
  humanized antibody
QASENIGNGLA

SEQ ID NO: 124 - protein, 11 aa, Artificial Sequence
  humanized antibody
LASEDIYSGIS

SEQ ID NO: 125 - protein, 11 aa, Artificial Sequence
  humanized antibody
QASEDIYSNLA

SEQ ID NO: 126 - protein, 11 aa, Artificial Sequence
  humanized antibody
QASEDIYSNLA

SEQ ID NO: 127 - protein, 11 aa, Artificial Sequence
  humanized antibody
QASEDIYSNLA

SEQ ID NO: 128 - protein, 11 aa, Artificial Sequence
  humanized antibody
QASENIYSSLA

SEQ ID NO: 129 - protein, 13 aa, Artificial Sequence
  humanized antibody
QSSQSVDGNNLLS

SEQ ID NO: 130 - protein, 11 aa, Artificial Sequence
  humanized antibody
QASQSIYSFLS

SEQ ID NO: 131 - protein, 11 aa, Artificial Sequence
  humanized antibody
QASQSIGYYLA

SEQ ID NO: 132 - protein, 11 aa, Artificial Sequence
  humanized antibody
QASQTISINLA

SEQ ID NO: 133 - protein, 11 aa, Artificial Sequence
  humanized antibody
QASQNIYSNLA

SEQ ID NO: 134 - protein, 13 aa, Artificial Sequence
  humanized antibody
QASQSVYNSNHLS

SEQ ID NO: 135 - protein, 11 aa, Artificial Sequence
  humanized antibody
QASQSISSYLS

SEQ ID NO: 136 - protein, 12 aa, Artificial Sequence
  humanized antibody
QASESISANYWS

SEQ ID NO: 137 - protein, 7 aa, Artificial Sequence
  humanized antibody
LASTLAS

SEQ ID NO: 138 - protein, 7 aa, Artificial Sequence
  humanized antibody
AASLLAS

SEQ ID NO: 139 - protein, 7 aa, Artificial Sequence
  humanized antibody
DASKLAS

SEQ ID NO: 140 - protein, 7 aa, Artificial Sequence
  humanized antibody
GASTLAS

SEQ ID NO: 141 - protein, 7 aa, Artificial Sequence
  humanized antibody
AASNLES

SEQ ID NO: 142 - protein, 7 aa, Artificial Sequence
  humanized antibody
GASTLAS

SEQ ID NO: 143 - protein, 7 aa, Artificial Sequence
  humanized antibody
RASTLAS

SEQ ID NO: 144 - protein, 7 aa, Artificial Sequence
  humanized antibody
DASTLAS

SEQ ID NO: 145 - protein, 7 aa, Artificial Sequence
  humanized antibody
DASDLAS

SEQ ID NO: 146 - protein, 7 aa, Artificial Sequence
  humanized antibody
DASNLAS

SEQ ID NO: 147 - protein, 7 aa, Artificial Sequence
  humanized antibody
AASDLES

SEQ ID NO: 148 - protein, 7 aa, Artificial Sequence
  humanized antibody
RASTLAS

SEQ ID NO: 149 - protein, 7 aa, Artificial Sequence
  humanized antibody
YASTLAS

SEQ ID NO: 150 - protein, 7 aa, Artificial Sequence
  humanized antibody
AASLLAS

SEQ ID NO: 151 - protein, 7 aa, Artificial Sequence
  humanized antibody
SASTLAS

SEQ ID NO: 152 - protein, 7 aa, Artificial Sequence
  humanized antibody
GASNLAS

SEQ ID NO: 153 - protein, 7 aa, Artificial Sequence
  humanized antibody
GASTLAS

SEQ ID NO: 154 - protein, 12 aa, Artificial Sequence
  humanized antibody
QNWWVIEHNGAA

SEQ ID NO: 155 - protein, 12 aa, Artificial Sequence
  humanized antibody
QSASYSTGPDWT

SEQ ID NO: 156 - protein, 12 aa, Artificial Sequence
  humanized antibody
QQGATTYNVDNV

SEQ ID NO: 157 - protein, 13 aa, Artificial Sequence
  humanized antibody
QCTYWNPDYIGGA

SEQ ID NO: 158 - protein, 12 aa, Artificial Sequence
  humanized antibody
LGGYSYSNTGPT

SEQ ID NO: 159 - protein, 15 aa, Artificial Sequence
  humanized antibody
LGVCTDISTDDLYNA

SEQ ID NO: 160 - protein, 12 aa, Artificial Sequence
  humanized antibody
LGVYTYSTDIHA

SEQ ID NO: 161 - protein, 12 aa, Artificial Sequence
  humanized antibody
LGVYTHISADNA

SEQ ID NO: 162 - protein, 13 aa, Artificial Sequence
  humanized antibody
QQGYYSGGTDNDV

SEQ ID NO: 163 - protein, 12 aa, Artificial Sequence
  humanized antibody
QGSYYSSSWYNV

SEQ ID NO: 164 - protein, 10 aa, Artificial Sequence
  humanized antibody
QCNYIIDYGA

SEQ ID NO: 165 - protein, 10 aa, Artificial Sequence
  humanized antibody
QSYYNSDSDA

SEQ ID NO: 166 - protein, 12 aa, Artificial Sequence
  humanized antibody
QQGYTEDNIDNT

SEQ ID NO: 167 - protein, 12 aa, Artificial Sequence
  humanized antibody
QGAVYSGNTEWA

SEQ ID NO: 168 - protein, 13 aa, Artificial Sequence
  humanized antibody
QGEFSCVSADCIA

SEQ ID NO: 169 - protein, 12 aa, Artificial Sequence
  humanized antibody
QCTYYDNNYGGA

SEQ ID NO: 170 - protein, 15 aa, Artificial Sequence
  humanized antibody
QSWYYSGSGSYHSWA

SEQ ID NO: 171 - protein, 107 aa, Homo sapiens [sequence omitted]

SEQ ID NO: 172 - protein, 329 aa, Homo sapiens
ASTKGPSVFPLAPSSKSTSGGTAALGCLVKDYFPEPVTVSWNSGALTSGVHTFPAVLQSSGLYSLSSVVTVPSSSLGTQTYICNVNHKPSNTKVDKKVEPKSCDKTHTCPPCPAPEAAGGPSVFLFPPKPKDTLMISRTPEVTCVVVDVSHEDPEVKFNWYVDGVEVHNAKTKPREEQYNSTYRVVSVLTVLHQDWLNGKEYKCKVSNKALPAPIEKTISKAKGQPREPQVYTLPPSREEMTKNQVSLTCLVKGFYPSDIAVEWESNGQPENNYKTTPPVLDSDGSFFLYSKLTVDKSRWQQGNVFSCSVMHEALHNHYTQKSLSLSPG

SEQ ID NO: 173 - protein, 123 aa, Artificial Sequence
  humanized antibody
EVQLLESGGRLVQPGTSLRLSCAVSGIDLSSYAMGWVRQAPGKGLEYVGVITSSATTYYASWAKGRFTISKTSSKNTLYLQMNSLRAEDTAVYFCARGGPGYSTNTHYAFDPWGQGTLVTVSS

SEQ ID NO: 174 - protein, 108 aa, Artificial Sequence
  Humanized antibody
DVQMTQSPSSLSASVGDRVTITCQASQSIYSFLSWYQQKPGQAPKLLIYAASDLESGVPSRFSGSGSGTDFTLTISSLQPEDFATYYCQSNYIIDYGAFGQGTKVVIK

SEQ ID NO: 175 - protein, 10 aa, Artificial Sequence
  Humanized antibody
QSNYIIDYGA

SEQ ID NO: 176 - protein, 118 aa, Artificial Sequence
  VR
QSLEESGGGLVKPEGSLTLTCKASGIDFSQDYYMCWVRQAPGKGLEWIACIYTGNDITYYASWAKGRFTVSKTSSTTVTLQMTSLTAADTATYFCARDGGANYYFKFWGQGTLVTVSS

SEQ ID NO: 177 - protein, 110 aa, Artificial Sequence
  VR
DIVMTQTPASVEAAVGGTVTIKCQASQSISNLLAWYQQKPGQPPKLLIYGASTLESGVPSRFKGSGSGTEFTLTISDLGSADAATYYCQNYAYSSGSWYSFGGGTEVVVK

SEQ ID NO: 178 - protein, 6 aa, Artificial Sequence
  CDR
QDYYMC

SEQ ID NO: 179 - protein, 17 aa, Artificial Sequence
  CDR
CIYTGNDITYYASWAKG

SEQ ID NO: 180 - protein, 10 aa, Artificial Sequence
  CDR
DGGANYYFKF

SEQ ID NO: 181 - protein, 11 aa, Artificial Sequence
  CDR
QASQSISNLLA

SEQ ID NO: 182 - protein, 7 aa, Artificial Sequence
  CDR
GASTLES

SEQ ID NO: 183 - protein, 12 aa, Artificial Sequence
  CDR
QNYAYSSGSWYS